European Patent Specification EP 4 077 359 B1, published March 18, 2026. Title: Genetically modified Clostridium strains and uses thereof. Applicant: Exomnis Biotech. The sequence listing filed with the application follows.

SEQUENCE LISTING (64 sequences)

SEQ ID NO: 1 - DNA, 34 bp, Artificial Sequence
  Cas9-F
tatagcggccgctcagtcacctcctagctgactc

SEQ ID NO: 2 - DNA, 48 bp, Artificial Sequence
  Cas9-R
ccggtctcacaagatggataagaaatactcaataggcttagatatcgg

SEQ ID NO: 3 - DNA, 46 bp, Artificial Sequence
  Prom-F
ccggtctcatggtcgtacactcccttttactatttaattatctatg

SEQ ID NO: 4 - DNA, 89 bp, Artificial Sequence
  sgRNA-R
tatagacgtcataaaaataagaagcctgcaaatgcaggcttcttatttttataaaaaaagcaccgactcggtgccactttttcaagttg

SEQ ID NO: 5 - DNA, 57 bp, Artificial Sequence
  Sag-LHA-F
tatataggtctcgggaaaataaagaaggacaagtattgctaaattcttatgatgtag

SEQ ID NO: 6 - DNA, 72 bp, Artificial Sequence
  Sag-LHA-R
tataggtctcgtctctgttaaccctcaaatttattatacctaataatcctttttaattattttcatgtacac

SEQ ID NO: 7 - DNA, 73 bp, Artificial Sequence
  Sag-RHA-F
tataggtctcggagatttacacagaggcccttagtatagtaattttatttgcagtaagtttctttattatagg

SEQ ID NO: 8 - DNA, 54 bp, Artificial Sequence
  Sag-RHA-R
tatataggtctcgtggcccaaagttcactaattttaactttaacaagaaacctg

SEQ ID NO: 9 - DNA, 89 bp, Artificial Sequence; identical to SEQ ID NO: 4
  Sag-SG-R

SEQ ID NO: 10 - DNA, 120 bp, Artificial Sequence
  Sag-SG-F
tatagtcgacgagttaatccatctgcaggagttttagagctagaaatagcaagttaaaataaggctagtccgttatcaacttgaaaaagtggcaccgagtcggtgctttttttataaaaa

SEQ ID NO: 11 - DNA, 28 bp, Artificial Sequence
  Upstream-F
tagcatcaggaggaacgaagataaaggc

SEQ ID NO: 12 - DNA, 26 bp, Artificial Sequence
  Junction-R
accgccacctacactaacactaacgc

SEQ ID NO: 13 - DNA, 36 bp, Artificial Sequence
  Downstream-R
ccataaatctctcaatatgtcaaagccatcaagtcc

SEQ ID NO: 14 - DNA, 56 bp, Artificial Sequence
  TreO-LHA-F
tatagacgtcgataagtcctattattattaaaatttcctataagaaaatattaatg

SEQ ID NO: 15 - DNA, 51 bp, Artificial Sequence
  TreO-LHA-R
ccggtctcggcagcattttcaactaatttaatatctccaataatattacgg

SEQ ID NO: 16 - RNA, 49 nt, Artificial Sequence
  TreO-RHA-F
ccggtctcagatttaaatttgtagaatttgcacgaagaaaataatactg

SEQ ID NO: 17 - DNA, 40 bp, Artificial Sequence
  TreO-RHA-R
tataggcgcgcccaataatttacaaggtatttaagataag

SEQ ID NO: 18 - DNA, 89 bp, Artificial Sequence; identical to SEQ ID NO: 4
  TreO-SG-R

SEQ ID NO: 19 - DNA, 120 bp, Artificial Sequence
  TreO-SG-F
ccgtcgacatacctccacagaacataaggttttagagctagaaatagcaagttaaaataaggctagtccgttatcaacttgaaaaagtggcaccgagtcggtgctttttttataaaaata

SEQ ID NO: 20 - DNA, 30 bp, Artificial Sequence
  Thl14YfkO-F
ccggtctcactgccaatagataaaataaag

SEQ ID NO: 21 - DNA, 42 bp, Artificial Sequence
  Thl14YfkO-R
ccggtctcaaatcataaaaataagaagcctgcaaatgcaggc

SEQ ID NO: 22 - DNA, 30 bp, Artificial Sequence
  CR2-TreO-F
gacttatttgggtttatttaaactaccccg

SEQ ID NO: 23 - DNA, 31 bp, Artificial Sequence
  CR2-TreO-R
tagcattggacattattgttaagcataagac

SEQ ID NO: 24 - DNA, 39 bp, Artificial Sequence
  pyrE-LHA-F
tatagacgtccctaaagaaggaaataatggcataagaat

SEQ ID NO: 25 - DNA, 52 bp, Artificial Sequence
  pyrE-LHA-R
ccggtctcaattattaaataattccccttatttcttctaaagtttgaatacc

SEQ ID NO: 26 - DNA, 49 bp, Artificial Sequence
  pyrE-RHA-F
ccggtctcaatttaaaaataaggagtgtctcaaaatagatttaattttg

SEQ ID NO: 27 - DNA, 47 bp, Artificial Sequence
  pyrE-RHA-R
tataggcgcgccagttgttccagatgttgatgtatactgcttatttg

SEQ ID NO: 28 - DNA, 43 bp, Artificial Sequence
  mIL2-F
ccggtctcataatttataaataaaaatcaccttttagaggtgg

SEQ ID NO: 29 - DNA, 54 bp, Artificial Sequence
  mIL2-R
ccggtctcaaaatttattatttatcatcatcatctttataatcttgaggacttg

SEQ ID NO: 30 - DNA, 89 bp, Artificial Sequence; identical to SEQ ID NO: 4
  pyrE-SG-R

SEQ ID NO: 31 - DNA, 120 bp, Artificial Sequence
  pyrE-SG-F
tagtcgacatagtaggaccagctatggggttttagagctagaaatagcaagttaaaataaggctagtccgttatcaacttgaaaaagtggcaccgagtcggtgctttttttataaaaata

SEQ ID NO: 32 - DNA, 38 bp, Artificial Sequence
  pyrE-ChR-R
ggagatatataatgcttcaagtaaatttatgtggtaag

SEQ ID NO: 33 - DNA, 37 bp, Artificial Sequence
  pyrE-ChR-F
ctccccataaataatcttgttttgacgctaatatagc

SEQ ID NO: 34 - DNA, 48 bp, Artificial Sequence
  Lspo-LHA-F
ccgacgtcgaaattgtgaaggaaaagacttaaaaatagtggcttatag

SEQ ID NO: 35 - DNA, 50 bp, Artificial Sequence
  Lspo-LHA-R
ccggtctcaggtcttaattattatctaatattccagcatcctttagcatc

SEQ ID NO: 36 - DNA, 41 bp, Artificial Sequence
  Lspo-RHA-F
ccggtctcaatggaagaaacaaagatcaatgttatcattgc

SEQ ID NO: 37 - DNA, 51 bp, Artificial Sequence
  Lspo-RHA-R
taggcgcgccctttccattatttatagtatacccaaatatattgtttatag

SEQ ID NO: 38 - DNA, 36 bp, Artificial Sequence
  bgaRL-F
ccggtctcactgccaatagataaaataaagtctgcc

SEQ ID NO: 39 - DNA, 53 bp, Artificial Sequence
  bgaRL-R
ccggtctcaccattttaccctcccaatacatttaaaataattatgtattcatg

SEQ ID NO: 40 - DNA, 89 bp, Artificial Sequence; identical to SEQ ID NO: 4
  LSpo0A-SG-R

SEQ ID NO: 41 - DNA, 120 bp, Artificial Sequence
  LSpo0A-SG-F
tagtcgacgtacaactcctttgtcactggttttagagctagaaatagcaagttaaaataaggctagtccgttatcaacttgaaaaagtggcaccgagtcggtgctttttttataaaaata

SEQ ID NO: 42 - DNA, 35 bp, Artificial Sequence
  spo0A-Chr-R2
cctgcagctgtatccggtatacaaataggagatag

SEQ ID NO: 43 - DNA, 29 bp, Artificial Sequence
  spo0A-Chr-F2
ggtcatttttaggtttattcccgtagacc

SEQ ID NO: 44 - DNA, 20 bp, Artificial Sequence
  pCB102-F
gcaaaatacattcgttgatg

SEQ ID NO: 45 - DNA, 25 bp, Artificial Sequence
  pCB102-R
ctttatttatgatttcatacttgac

SEQ ID NO: 46 - DNA, 23 bp, Artificial Sequence
  BM1
gttaacagagatttacacagagg

SEQ ID NO: 47 - DNA, 23 bp, Artificial Sequence
  BM2
gcagccctccactcccatggagg

SEQ ID NO: 48 - DNA, 46 bp, Artificial Sequence
  pyrE-BM2-LHA
ccggtctcactgcttaaataattccccttatttcttctaaagtttg

SEQ ID NO: 49 - DNA, 64 bp, Artificial Sequence
  pyrE-BM2-RHA
ccggtctcagcagccctccactcccatggaggatttaaaaataaggagtgtctcaaaatagatt

SEQ ID NO: 50 - DNA, 53 bp, Artificial Sequence
  bgaL-RbEspo0A-R
ccggtctcaccatcttgttgttacctccttagcagggtgctgccaagggcatc

SEQ ID NO: 51 - DNA, 62 bp, Artificial Sequence
  PSpoIIAA-SG1-F
tagtcgacggatttggatgagtaaaaaggttttagagctagaaatagcaagttaaaataagg

SEQ ID NO: 52 - DNA, 89 bp, Artificial Sequence; identical to SEQ ID NO: 4
  sgRNA-Uni-R

SEQ ID NO: 53 - DNA, 52 bp, Artificial Sequence
  spoIIAA-LHA-F
tatagacgtcgagtctataaatttatgaattttaaaatattttttaggtaag

SEQ ID NO: 54 - DNA, 47 bp, Artificial Sequence
  spoIIAA-LHA-R
ccggtctcagcaggtaaaaattttttatattgattattctagaacac

SEQ ID NO: 55 - DNA, 43 bp, Artificial Sequence
  spoIIAA-RHA-F
ccggtctcaatgtatttaaaatttgataaaaaagcagacaaac

SEQ ID NO: 56 - DNA, 31 bp, Artificial Sequence
  spoIIAA-RHA-R
ggcgcgcctttagttcccttccccttttctg

SEQ ID NO: 57 - DNA, 53 bp, Artificial Sequence
  bgaL-RbEspoIIAA-R
ccggtctcaacatcttgttgttacctccttagcagggtgctgccaagggcatc

SEQ ID NO: 58 - DNA, 27 bp, Artificial Sequence
  Chr-spoIIAA-F
ccacttgggtatgttggaatagctgcc

SEQ ID NO: 59 - DNA, 27 bp, Artificial Sequence
  Chr-spoIIAA-R
ccagatcttgcctcttccataagttcc

SEQ ID NO: 60 - DNA, 1349 bp, Artificial Sequence
  BgaR-bglA-RbE sequence
ctgccaatagataaaataaagtctgccacaattgtggcagactttattttatctattgatttatttcattttttaatttatatacttggtttatttacttgattatttctgtaatttagtggagacattgaaaaatgttttgaaaaagtttttgaaaataacagggagtcactataacctacactacttgcgacttctcctataggaagtttagtgctttttaataaaagggtggctttgtacattctaaggtttattaaatatctttgaggagaaattccaaggttttttatgaacattttatataaataacttctacttaagttcacataatcagcaatttcttgaacagttatgctatgcatgtaattagaattaatgaaattaagagcatcttgaatatatgtgtgtaattccttatctttgtattcaaaaggttttgggaattcttctataagtgcgtacaataatgagtaaagttcttttagtaatagtatgtcatcagatcttgaaggattataagtttttgatatttcgcacatatttaatattatctgtggaatttttgagttttcttcacaattagcaacacaggagttagtaatagaagttctatttaaatactcattagcatttgaaccactaaatcctatccagtagtattcccaaggatcatcaatagaagccacatactcaacttgcataccttttagtagtataaaaatatcaccttgttttaagttatataccttaccattaaatttaaaagttccatatcccttagttacgtaatgaataacagcatttttcaatacttcatagttatatcctaatcctggtataccttgttctataccacattcatctacattcatttcaaagttttctttaacatactttttccacaatatttgcatttctacctcctaacctataaaattagccaattttatagtagtcttatattaaacatttacatgagagctttgcaaagcagtttatcaacataaaagctttttattttaaaataaattcttctaaatataagaatattttaaagaaatatctttatatattagttattaaaatttataagattataagaaacattataacatattttagaactttttaactattctaaaagattaatttacatattaacatttaattatgggtaaaaactattttgaaaaatgatttatatggaattatgtttcttaaatatacaatcatgtttcatgaatacataattattttaaatgtattgaatacgactcactataggtgataccagcatcgtcttgatgcccttggcagcaccctgctaaggaggtaacaacaagatg

SEQ ID NO: 61 - DNA, 580 bp, Artificial Sequence
  Synthesized module F2 for pPME-100 derivative plasmids
tggtcgtacactcccttttactatttaattatctatgttaaatgattaacgtgctcatttatattttaacaaacttttcacatgaagttaagttttttagaaaattatttatattttatattttctcattatactttctgctgacttatctagatttatatttagtcccttgccttgcctacaagggatttcctattcctttcatttacaattcatacgtataaaatccaaatttttcttgacatttatacacataaatattatgatttatataggtaatcgctttcataaaatatattacccttaggaaatcaaatgattataagtcatatatgaaaacgttatatataattgatatgtttacatttgtaacttagatttctctttgatttccacatatataaatcttaaggaggagttttcgtcgacatagtaggaccagctatggggttttagagctagaaatagcaagttaaaataaggctagtccgttatcaacttgaaaaagtggcaccgagtcggtgctttttttataaaaataagaagcctgcatttgcaggcttcttatttttatgacgtc

SEQ ID NO: 62 - DNA, 828 bp, Artificial Sequence
  Thl14-YfkO
ttagcatatgcataagtttaatttttttgttaaaaaatattaaactttgtgttttttttaacaaaatatattgataaaaataataatagtgggtataattaagttgttagagaaaacgtaataaaataaaggaggtttatatatatgacagaacaaagcaagaaacaagaaatactagatgcttttcagtttagacatgcaacaaaagagtttgatccagataggaaaatatcagatgaagatttccaattcatacttgaagctggtagattatcaccatcttctgtaggtttagaaccttggcaatttgtagttgtacaaaataaagaactaagagaaaagttaagacaagtttcttggggagctcaaggacaattaccaactgcatctcattttgtacttttattaggtagaacagctaaagaaatgagaagagatagtggatatgtagctgatcaattgaaacatgttaagaaaatgcctgaagatataatagaaaatatgctaaaagaagatggagttttagaaagttttcaagatggtgattttcacttgtatgaatcagatagagcaatgtttgattgggttagtaaacaaacttacattgcattagcaaatatgatgactgcagctgctttaataggaattgattcttgtccaattgaaggatttaactatgacaaagtacatgacatacttgagaaagaaggtgtattagaagatggaagatttgacatatcagtaatggcagcttttggatatagagtaaaagaacctagacccaaaactagaagagctttagatcaaattgtaaaatgggttgaataa

SEQ ID NO: 63 - DNA, 808 bp, Artificial Sequence
  PfdxnprM3-mIL2-Flag
taatttataaataaaaatcaccttttagaggtggtttttttatttataaattagtgtagtagcctgtgaaataagtaaggaaaaaaaagaagtaagtgttatatatgatgattattttgtagatgtagataggataatagaatccatagaaaatataggttatacagttatataaaaattactttaaaaattaataaaaacatggtaaaatataaatcgtataaagttgtgtaatttttaaggaggtgtgttacatatgaaaagtaaaaaattattagctacagtgctaagtgctgtaatcactctttctactgtttctgcagtttatgctgctccaacttctagttcaacttcaagttctacagctgaagcacaacaacagcaacaacagcaacaacaacagcaacaacatcttgaacaactattaatggatctacaagaacttctatctagaatggaaaattatagaaaccttaaactaccaagaatgctaacatttaaattttatttaccaaaacaagcaacagaattaaaagatcttcagtgtctcgaagatgaacttggtcctctacgtcatgttctagatttaactcaaagtaaaagttttcaattggaagatgcagaaaattttataagtaatattagagtaactgttgtaaaactaaagggatctgataacacttttgaatgtcaattcgatgatgaatcagctactgttgtagattttctaagaaggtggatagcattctgtcaaagtatcatatctacaagtcctcaagattataaagatgatgatgataaataataa

SEQ ID NO: 64 - DNA, 56 bp, Artificial Sequence
  fdx-RsE (RbE)
ggtgataccagcatcgtcttgatgcccttggcagcaccctgctaaggaggcaacaa